European Patent Application EP 4 327 830 A1, published February 28, 2024. Title: A METHOD OF MODIFYING AN ORGANIC CYTOTOXIN FOR USE AS A PAYLOAD IN AN ANTIBODY-DRUG CONJUGATE AND MODIFIED ORGANIC CYTOTOXINS DERIVED THEREFROM. Applicant: Cyano Biotech GmbH. Application EP, filed August 27, 2022. The sequence listing filed with the application follows.

SEQUENCE LISTING (3 sequences)

SEQ ID NO: 1 - protein, 8 aa, Amanita sp.
  VARIANT 1: note = Ile, Hyile or Dihyile
  VARIANT 2: note = Trp or Hytrp
  VARIANT 7: note = Asn or Asp
  VARIANT 8: note = Pro or Hypro
  CROSSLNK 1..8: note = peptide bond
  CROSSLNK 2..6: note = sulfoxide bridge
IWGIGCJP

SEQ ID NO: 2 - protein, 7 aa, synthetic construct
  SITE 1: note = D-Ala
  SITE 2: note = Azidonorvaline (Aznva)
  SITE 3: note = D-Asp
  SITE 5: note = Adda
  SITE 6: note = D-Glu
  SITE 7: note = Mdha
  CROSSLNK 1..7: note = peptide bond
AXDRXEX

SEQ ID NO: 3 - protein, 7 aa, synthetic construct
  SITE 1: note = D-Ala
  SITE 2: note = Propargyltyrosine (Prtyr)
  SITE 3: note = D-Asp
  SITE 5: note = Adda
  SITE 6: note = D-Glu
  SITE 7: note = Mdha
  CROSSLNK 1..7: note = peptide bond
AXDRXEX